European Patent Application EP 4 234 572 A1, published August 30, 2023. Title: Proteoglycan conjugate and application thereof. Applicant: SHANGHAI REINOVAX BIOLOGICS CO., LTD SHANGHAI MICRODOM BIOTECH CO., LTD. The sequence listing filed with the application follows.

SEQUENCE LISTING (8 sequences)

SEQ ID NO: 1 - protein, 487 aa, Artificial Sequence
  TTD-1
MQYIKANSKFIGITELKKLESKINKVFSTPIPFSYSKNLDCWVDNEEDIDVILKKSTILNLDINNDIISDISGFNSSVITYPDAQLVPGINGKAIHLVNNESSEVIVHKAMDIEYNDMFNNFTVSFWLRVPKVSASHLEQYGTNEYSIISSMKKHSLSIGSGWSVSLKGNNLIWTLKDSAGEVRQITFRDLPDKFNAYLANKWVFITITNDRLSSANLYINGVLMGSAEITGLGAIREDNNITLKLDRCNNNNQYVSIDKFRIFCKALNPKEIEKLYTSYLSITFLRDFWGNPLRYDTEYYLIPVASSSKDVQLKNITDYMYLTNAPSYTNGKLNIYYRRLYNGLKFIIKRYTPNNEIDSFVKSGDFIKLYVSYNNNEHIVGYPKDGNAFNNLDRILRVGYNAPGIPLYKKMEAVKLRDLKTYSVQLKLYDDKNASLGLVGTHNGQIGNDPNRDILIASNWYFNHLKDKILGCDWYFVPTDEGWTND

SEQ ID NO: 2 - protein, 476 aa, Artificial Sequence
  TTD-2
GITELKKLESKINKVFSTPIPFSYSKNLDCWVDNEEDIDVILKKSTILNLDINNDIISDISGFNSSVITYPDAQLVPGINGKAIHLVNNESSEVIVHKAMDIEYNDMFNNFTVSFWLRVPKVSASHLEQYGTNEYSIISSMKKHSLSIGSGWSVSLKGNNLIWTLKDSAGEVRQITFRDLPDKFNAYLANKWVFITITNDRLSSANLYINGVLMGSAEITGLGAIREDNNITLKLDRCNNNNQYVSIDKFRIFCKALNPKEIEKLYTSYLSITFLRDFWGNPLRYDTEYYLIPVASSSKDVQLKNITDYMYLTNAPSYTNGKLNIYYRRLYNGLKFIIKRYTPNNEIDSFVKSGDFIKLYVSYNNNEHIVGYPKDGNAFNNLDRILRVGYNAPGIPLYKKMEAVKLRDLKTYSVQLKLYDDKNASLGLVGTHNGQIGNDPNRDILIASNWYFNHLKDKILGCDWYFVPTDEGWTND

SEQ ID NO: 3 - protein, 451 aa, Artificial Sequence
  TTD-3
KNLDCWVDNEEDIDVILKKSTILNLDINNDIISDISGFNSSVITYPDAQLVPGINGKAIHLVNNESSEVIVHKAMDIEYNDMFNNFTVSFWLRVPKVSASHLEQYDTNEYSIISSMKKYSLSIGSGWSVSLKGNNLIWTLKDSAGEVRQITFRDLSDKFNAYLANKWVFITITNDRLSSANLYINGVLMGSAEITGLGAIREDNNITLKLDRCNNNNQYVSIDKFRIFCKALNPKEIEKLYTSYLSITFLRDFWGNPLRYDTEYYLIPVAYSSKDVQLKNITDYMYLTNAPSYTNGKLNIYYRRLYSGLKFIIKRYTPNNEIDSFVRSGDFIKLYVSYNNNEHIVGYPKDGNAFNNLDRILRVGYNAPGIPLYKKMEAVKLRDLKTYSVQLKLYDDKDASLGLVGTHNGQIGNDPNRDILIASNWYFNHLKDKTLTCDWYFVPTDEGWTND

SEQ ID NO: 4 - DNA, 1458 bp, Artificial Sequence
  TTD-4
cagtatataaaagcaaattctaaatttataggtataactgaactaaaaaaattagaatcaaaaataaacaaagttttttcaacaccaattccattttcttattctaaaaatctggattgttgggttgataatgaagaagatatagatgttatattaaaaaagagtacaattttaaatttagatattaataatgatattatatcagatatatctgggtttaattcatctgtaataacatatccagatgctcaattggtgcccggaataaatggcaaagcaatacatttagtaaacaatgaatcttctgaagttatagtgcataaagctatggatattgaatataatgatatgtttaataattttaccgttagcttttggttgagggttcctaaagtatctgctagtcatttagaacaatatggcacaaatgagtattcaataattagctctatgaaaaaacatagtctatcaataggatctggttggagtgtatcacttaaaggtaataacttaatatggactttaaaagattccgcgggagaagttagacaaataacttttagggatttacctgataaatttaatgcttatttagcaaataaatgggtttttataactattactaatgatagattatcttctgctaatttgtatataaatggagtacttatgggaagtgcagaaattactggtttaggagctattagagaggataataatataacattaaaactagatagatgtaataataataatcaatacgtttctattgataaatttaggatattttgcaaagcattaaatccaaaagagattgaaaaattatacacaagttatttatctataacctttttaagagacttctggggaaaccctttacgatatgatacagaatattatttaataccagtagcttctagttctaaagatgttcaattgaaaaatataacagattatatgtatttgacaaatgcgccatcgtatactaacggaaaattgaatatatattatagaaggttatataatggactaaaatttattataaaaagatatacacctaataatgaaatagattcttttgttaaatcaggtgattttattaaattatatgtatcatataacaataatgagcacattgtaggttatccgaaagatggaaatgcctttaataatcttgatagaattctaagagtaggttataatgccccaggtatccctctttataaaaaaatggaagcagtaaaattgcgtgatttaaaaacctattctgtacaacttaaattatatgatgataaaaatgcatctttaggactagtaggtacccataatggtcaaataggcaacgatccaaatagggatatattaattgcaagcaactggtactttaatcatttaaaagataaaattttaggatgtgattggtactttgtacctacagatgaaggatggacaaatgat

SEQ ID NO: 5 - DNA, 1428 bp, Artificial Sequence
  TTD-5
ggaattacagaattaaaaaagctggagagtaagataaataaggtttttagcacgcctatacctttctcgtatagtaaaaaccttgactgctgggtggataacgaagaggacatcgacgtcatattgaaaaaatcgactattttaaatttagacattaacaatgacattatttcggacatttcaggctttaactcatcagtaataacttatcctgacgcacaattggtccctggaatcaacggtaaagccatccatctggtgaacaacgaaagttccgaagtgattgtccataaagctatggacattgagtataacgatatgtttaataatttcactgtgagtttttggctgcgtgtccctaaagtatctgccagtcacttagagcaatatggtacgaacgaatactcgataatttcatctatgaaaaaacatagcttgtcaatcggctcaggctggtccgtctcactgaagggcaataatcttatctggaccctgaaggactctgcgggtgaagtacggcagatcacgtttagagatcttccggataaatttaacgcttatttagcgaacaaatgggtctttatcactatcacaaatgatcgtctgtcgagcgccaacctttatattaacggagtactgatgggtagtgctgagattaccggacttggagcgattcgggaagacaacaacatcacccttaaacttgatcgttgtaacaataataatcagtacgtgagcatcgacaagtttcggatattttgtaaggcgttaaatccgaaggaaattgaaaaattatatacatcgtatctgtcaatcactttcttgcgggatttctgggggaatcctcttcggtatgataccgaatactatcttatacctgtggcatctagtagtaaggatgtacagttgaagaacattacagattatatgtatcttaccaatgcacccagttacacaaacggcaagttaaatatctattatcgccggctttataacggtctgaaattcatcataaaaagatacactcccaacaacgagatagattcttttgtcaagagcggagacttcattaagttatatgtcagctacaacaacaatgagcacatagttggctacccaaaggacggaaacgcgtttaacaacctggatcgtatactgcgggtgggctataacgcgcctgggattcccttgtataaaaagatggaagcagtaaaattgcgcgacttgaagacgtactccgtacaacttaaactttacgacgacaaaaatgcgagtcttggattggttggtacgcacaacggacagatcgggaatgatccgaaccgtgacatcttaattgcatcaaattggtactttaatcatttgaaagacaaaatccttggctgcgattggtattttgttccgactgatgaggggtggacgaacgac

SEQ ID NO: 6 - DNA, 1353 bp, Artificial Sequence
  TTD-6
aaaaaccttgactgctgggtggataacgaagaggacatcgacgtcatattgaaaaaatcgactattttaaatttagacattaacaatgacattatttcggacatttcaggctttaactcatcagtaataacttatcctgacgcacaattggtccctggaatcaacggtaaagccatccatctggtgaacaacgaaagttccgaagtgattgtccataaagctatggacattgagtataacgatatgtttaataatttcactgtgagtttttggctgcgtgtccctaaagtatctgccagtcacttagagcaatatggtacgaacgaatactcgataatttcatctatgaaaaaacatagcttgtcaatcggctcaggctggtccgtctcactgaagggcaataatcttatctggaccctgaaggactctgcgggtgaagtacggcagatcacgtttagagatcttccggataaatttaacgcttatttagcgaacaaatgggtctttatcactatcacaaatgatcgtctgtcgagcgccaacctttatattaacggagtactgatgggtagtgctgagattaccggacttggagcgattcgggaagacaacaacatcacccttaaacttgatcgttgtaacaataataatcagtacgtgagcatcgacaagtttcggatattttgtaaggcgttaaatccgaaggaaattgaaaaattatatacatcgtatctgtcaatcactttcttgcgggatttctgggggaatcctcttcggtatgataccgaatactatcttatacctgtggcatctagtagtaaggatgtacagttgaagaacattacagattatatgtatcttaccaatgcacccagttacacaaacggcaagttaaatatctattatcgccggctttataacggtctgaaattcatcataaaaagatacactcccaacaacgagatagattcttttgtcaagagcggagacttcattaagttatatgtcagctacaacaacaatgagcacatagttggctacccaaaggacggaaacgcgtttaacaacctggatcgtatactgcgggtgggctataacgcgcctgggattcccttgtataaaaagatggaagcagtaaaattgcgcgacttgaagacgtactccgtacaacttaaactttacgacgacaaaaatgcgagtcttggattggttggtacgcacaacggacagatcgggaatgatccgaaccgtgacatcttaattgcatcaaattggtactttaatcatttgaaagacaaaatccttggctgcgattggtattttgttccgactgatgaggggtggacgaacgac

SEQ ID NO: 7 - protein, 36 aa, Artificial Sequence
  The amino acid sequence 07 of the translocation region
MQYIKANSKFIGITELKKLESKINKVFSTPIPFSYS

SEQ ID NO: 8 - protein, 25 aa, Artificial Sequence
  The amino acid sequence 08 of the translocation region
GITELKKLESKINKVFSTPIPFSYS